European Patent Application EP 4 582 551 A1, published July 9, 2025. Title: Method of identifying lipase. Applicant: 花王株式会社. The sequence listing filed with the application follows.

SEQUENCE LISTING (57 sequences)

SEQ ID NO: 1 - DNA, 807 bp, Thermomyces lanuginosus
  source 1..807: mol_type = genomic DNA
gaagtgagccaagatttatttaaccagtttaacctgtttgcgcaatattctgcagcggcttattgcggaaaaaataacgatgccccggcaggaacaaatatcacatgcacaggcaacgcttgtccggaagttgaaaaagcggatgctacatttctttactcatttgaagatagcggcgtgggagatgtcacaggctttctggcccttgataacacaaacaaactgatcgtgctgtcatttagaggaagccgctctatcgaaaactggatcggcaaccttaactttgatctgaaagaaatcaacgatatctgctcaggctgtagaggacatgatggctttacatcaagctggagaagcgtcgcggatacattacgccagaaagttgaagatgctgtgagagaacatccggattatcgcgttgtgtttacaggacattctctgggcggagcccttgcaacagttgctggagctgatctgagaggcaacggatacgatatcgatgtcttttcatacggagctccgagagttggcaaccgcgcctttgcagaatttcttacagtgcaaacaggcggaacactgtaccgcatcacacatacaaacgatattgtcccgagactgccgccgcgcgaatttggatattctcattcttcaccggaatattggatcaaatcaggcacacttgtcccggttacacgcaacgatatcgttaaaatcgaaggaatcgatgccacaggcggaaataaccagccgaacatcccggatattccggcacatttatggtattttggactgattggcacatgtctt

SEQ ID NO: 2 - protein, 269 aa, Thermomyces lanuginosus [sequence omitted]

SEQ ID NO: 3 - DNA, 876 bp, Cedecea sp.
  source 1..876: mol_type = genomic DNA
atgtctacatcactgaaatatccgattgtccttgttcatggcctgcttggatttgataaaattggcggaatctacccgtacttttacggaatcaaagaagcgctggaaaaagcaggcgcgaaagtgtatatcgcaacattaagcgcgctgaattctaacgaaatgagaggagaacaattactggaatttgtgcgcaaagtccaggctgaaacaggcgcagcgaaagttaatcttattggccattctcaaggaccgttagcttgcagatatgtggctgccacacatccggatctgatcgcctcagttacaagcgtgaatggcgtcaaccatggatcagaagttgctgatcttgtgagactggcccttaaaccgggacgcttaccggaatcaattgcaaatgcagcgctgagcgcgtttggccaacttttatctgctttagctggagaaccgagactgcctcagtcaggcgtggatgcacttgatgcgttaacaagcgaaggagtcgctgcctttaacaaaaaatatccgcaaggattacctgcagaatggggcggacagggaaaagaactggataacggagtctactactacagctggtctggaattatcgattataacccgctgcatcaaggcatgaataacctggatccgcttcatgttgctatgcttgcctttagcatcctgtttacaaacgaaagatttcagaacgatggcctggtgggacgctattcaagccatcttggcaaagtcattggatctgattattcaatggatcatgttgatgcgatcaatcaactggctggagttgtggccaataacacagatccggtcaaactttatgttgatcatttagcaagactgcaggcgaaaggctta

SEQ ID NO: 4 - protein, 292 aa, Cedecea sp.
MSTSLKYPIVLVHGLLGFDKIGGIYPYFYGIKEALEKAGAKVYIATLSALNSNEMRGEQLLEFVRKVQAETGAAKVNLIGHSQGPLACRYVAATHPDLIASVTSVNGVNHGSEVADLVRLALKPGRLPESIANAALSAFGQLLSALAGEPRLPQSGVDALDALTSEGVAAFNKKYPQGLPAEWGGQGKELDNGVYYYSWSGIIDYNPLHQGMNNLDPLHVAMLAFSILFTNERFQNDGLVGRYSSHLGKVIGSDYSMDHVDAINQLAGVVANNTDPVKLYVDHLARLQAKGL

SEQ ID NO: 5 - DNA, 861 bp, Proteus vulgaris
  source 1..861: mol_type = genomic DNA
atgagtacgacttatccgattgttttggtacacggactctccggctttgatgacatagtcggctacccttatttttacggaatcgcagacgcactggagaaggacggacataaagtgttcacggcctcgctttcggcttttaacagcaatgaagtccgcggagagcagctttgggaatttgttcaaaaaattctgaaggaaacaaaagcgaagaaagttaacctgatcggccattcacaaggaccgcttgcctgcaggtacgtggcagcaaagcatgcaaaaagcatagcatctgttacatctgtcaacggagtgaatcacggcagtgaaattgcggatttggtgcgccggatcatgagaaaagacagcgtaccagagtacattgctgatgcggtcatgaaagcgatcggtaccatcattagcaccttttccgggaaccgaggaaatccgcaggatgccattgccgcgttagaggctttaactacagaaaatgtgatggaattcaataaaaaatatcctcaaggtcttccagccattcgcggcggcgaaggcaaggaagtggtcaatggtgttcattattattcatttggttcttatattcaaggcctcatcgcgggagaaaaagggaatcttttggatcccacacacgctgcgatgcgtgtattgtcagcgtttttctctgaaagagaaaacgacggcttagtaggcagaacgagcatgcggttaggaaaactgattaaagatgattatgcagaggatcatttagatatggtgaaccaggttgctgggctcgtcgggcgtggggaagatatcattgcaatatatacaaatcatgccaatttcctggcttcaaaaaagcta

SEQ ID NO: 6 - protein, 287 aa, Proteus vulgaris
MSTTYPIVLVHGLSGFDDIVGYPYFYGIADALEKDGHKVFTASLSAFNSNEVRGEQLWEFVQKILKETKAKKVNLIGHSQGPLACRYVAAKHAKSIASVTSVNGVNHGSEIADLVRRIMRKDSVPEYIADAVMKAIGTIISTFSGNRGNPQDAIAALEALTTENVMEFNKKYPQGLPAIRGGEGKEVVNGVHYYSFGSYIQGLIAGEKGNLLDPTHAAMRVLSAFFSERENDGLVGRTSMRLGKLIKDDYAEDHLDMVNQVAGLVGRGEDIIAIYTNHANFLASKKL

SEQ ID NO: 7 - DNA, 879 bp, unidentified
  source 1..879: mol_type = genomic DNA
atgtcggcttctagcctgaaatttccgatcgtgctcgttcacggcctgttaggttttgataaaatcggcggaatctatccttatttttacggcattaaagaggcgcttgaaaaagcgggagcgaaggtttatattgcgacactttctgctttgaacagcaatgaacttcgcggagaacagttgttggaatttgtcagaaaagttcaggcagaaacaggcgcggcaaaagtgaatcttattggacactcacaaggcccgctggcatgccgctatgtggcggccactcatccggagctgattgcatctgtcacgtcggtaaacggcgtcaatcatgggagtgaagtggctgatcttgtaagattggctctgacaccgggacgactccctgaatccatagccaatgcagcgatgtcagcattcggacagttactctcggcattggccgggtcaccccgtcttccacagtcaggaattgaagcattagaagctttaacgtctgaaggagttgccgcctttaacaataaatatccgcaaggactgcctgctgaatggggcggtgagggcaaagaattggtaaacggtgtatattattactcttggagcggtgtgattgattataaccctcttcatcagggggcaaacaacttagacccgcttcatgtcgcaatgctggctttctccatcctgtttactaatgagcgttttcaaaatgacgggcttgtcggccggtactcctcacacctaggaaaagtcattgggagtgattacagcatggatcatgttgatgcgatcaatcaattagccggtgttgtcgctaataacaccgacccagttcaattattcgtggagcatgtggcgaggctgaagagcaagggcctc

SEQ ID NO: 8 - protein, 293 aa, unidentified
MSASSLKFPIVLVHGLLGFDKIGGIYPYFYGIKEALEKAGAKVYIATLSALNSNELRGEQLLEFVRKVQAETGAAKVNLIGHSQGPLACRYVAATHPELIASVTSVNGVNHGSEVADLVRLALTPGRLPESIANAAMSAFGQLLSALAGSPRLPQSGIEALEALTSEGVAAFNNKYPQGLPAEWGGEGKELVNGVYYYSWSGVIDYNPLHQGANNLDPLHVAMLAFSILFTNERFQNDGLVGRYSSHLGKVIGSDYSMDHVDAINQLAGVVANNTDPVQLFVEHVARLKSKGL

SEQ ID NO: 9 - DNA, 867 bp, Buttiauxella brennerae
  source 1..867: mol_type = genomic DNA
atgtgcacaaaatacccagtcgttctcgttcatggctggagcggcttttctacgattcttggctatccatattatttcggtgtgaaggaagcgcttgagaagaagggagcagatgtgtatacggcgtctttgtccggagtcaatacagacgatgtcagaggtgaacagctgtgggattttattcaggatgtaaagcgaaaaagcggcaaagataaagtgaacctgatcggccattcacaaggcgcgttggactgtcggtatgtggctgctgtttatccgcattctgtcgcttcagtaactagcgttgatggcgcaaatcacggctcagagtccgctgatgcgcttagagcagcctatgaaccggggtcttgcaaagaaggatttgtcgcgctagcagtgaatgcatttgaaaaagccatcgccttcctttcgggacatccgtttgagcccgaagactttatcgcttctttaaattccctgacgacagaaggggtacaggcgtttaacgaaaaatatcctcaaggtctccctgaagtgtggggaggagaaggccctgaggttgtcaacggtatttattactacagctggagtggcattataaaagacgggatatgcgaacaaggattgaatgagctggatccgcttcacttatggatgaaacatggggccaaaacatttgtgaatgaagtagatcaaaatgacgggttggtaggtaggtacagttcacacctcggaaaagtgatttgttcagattatagcatggatcatttagatgcaatcaatcagttagccggaatccgtacaaacaccgttaacgttattgatctgtacactgaccatcttgacttcttacgctcgaagggtgtc

SEQ ID NO: 10 - protein, 289 aa, Buttiauxella brennerae
MCTKYPVVLVHGWSGFSTILGYPYYFGVKEALEKKGADVYTASLSGVNTDDVRGEQLWDFIQDVKRKSGKDKVNLIGHSQGALDCRYVAAVYPHSVASVTSVDGANHGSESADALRAAYEPGSCKEGFVALAVNAFEKAIAFLSGHPFEPEDFIASLNSLTTEGVQAFNEKYPQGLPEVWGGEGPEVVNGIYYYSWSGIIKDGICEQGLNELDPLHLWMKHGAKTFVNEVDQNDGLVGRYSSHLGKVICSDYSMDHLDAINQLAGIRTNTVNVIDLYTDHLDFLRSKGV

SEQ ID NO: 11 - DNA, 870 bp, Pseudomonas frederiksbergensis
  source 1..870: mol_type = genomic DNA
atgaatatggacgcgtcaacgcaatatccgatagtgcttgttcacggtttgtttggcttcgatacaatcggcggatacccttatttttttgaaatcaaagaagcgcttgaaagggcgggagcaaaagtgtacgctgtcaatattccagcggttaacggcaatgaagagcggggagaaaaactattggagcatgtgaaccgcattcttcgcgaaacaggcgccgccaaggtcaacctgatcggacattcacaaggcccgctggcagcccgatacgtggcagctctgcatccgcaaaaagtagccagtgtcactagtgtgagctgtcccaatcatggatcggaaattgctgatcagcttcataaagcgctgacgcctggcgagctgccagaagcagttgttctggcattattcgccgctgtcggcattttcatctccctaatatccgggcatcctgaaaatccgcaggacgcgcgtgctgcctttgcatcactcacctctgaaggtcttgcggcttttaacaaaaagtatccccagggggttccgaaacattggggtggcgacgggaatgagattgaaaacggagtttattattactcttggtcaggtattgttcagaattttcaatccttacagccactggatccgagccacttaaactgcattgtgctcagtaagctgttttataaagagaaacacgcgaatgacggacttgtcggacaaaacagctctcatttggggaaagtaatcagatctgattatccgatggatcattttgatgctgtaaatcaaatggcagggattacaagctggaatgtctcgcctgtacacctctatttggaacacgcagcaagattaaaggataaaggctta

SEQ ID NO: 12 - protein, 290 aa, Pseudomonas frederiksbergensis
MNMDASTQYPIVLVHGLFGFDTIGGYPYFFEIKEALERAGAKVYAVNIPAVNGNEERGEKLLEHVNRILRETGAAKVNLIGHSQGPLAARYVAALHPQKVASVTSVSCPNHGSEIADQLHKALTPGELPEAVVLALFAAVGIFISLISGHPENPQDARAAFASLTSEGLAAFNKKYPQGVPKHWGGDGNEIENGVYYYSWSGIVQNFQSLQPLDPSHLNCIVLSKLFYKEKHANDGLVGQNSSHLGKVIRSDYPMDHFDAVNQMAGITSWNVSPVHLYLEHAARLKDKGL

SEQ ID NO: 13 - DNA, 885 bp, Entomomonas sp.
  source 1..885: mol_type = genomic DNA; note = Entomomonas sp. F2A
atggactcaaaatcaaacaatagtgcgattatcaattcaactaagtacccaattttgcttgtccacgggttgttcggctttgaaaaaattgccggatacccctacttttataaaatagatgagctgctgcgacagcaaggagcgaatgtattcacacctgttgtatcggctgcaaatacaacgaaaaacagaggggaacagcttcttttgcagattaaacaaatccttgatcttactaaagcagacaaagtaaacctcattggccattctcacggagcgcttacggcacgttatgtggcagcctgctacccagagcttgttgcttcagtcacctcggtgaatggtgtaaatcatggttcagaaattgctgacgtgatgttaaaggttctgaagaacaaactttcatcatcaatagccaacaagctgatctctcactttgtcaacagcgttaccctgttatcaacaaagcggcatctgcctcaggattttatcggcgctttgaactgcctgtctactgaaggagttaaacattttaataaccaatatccgcagggcattccgacaacatgggggggagaaggcttagagctcgaaaacaacaatgtgtattattacagctggagcggtatcttaaatacgatcccgattacgctgtcaaataaattctccttactcagtttgagctcccgctattttgtgaaagaacttcaacaaaatgacggcctagtcggccgtttttcctctcatttaggtaaggtcatccgctctgattatccgatggatcatgcagcggcggttaatcagatcaggggaaaatgtaatgcatccattgatcctacagccttatatattgagcatttacaaagattggctctcaaagggcta

SEQ ID NO: 14 - protein, 295 aa, Entomomonas sp.
  source 1..295: note = Entomomonas sp. F2A
MDSKSNNSAIINSTKYPILLVHGLFGFEKIAGYPYFYKIDELLRQQGANVFTPVVSAANTTKNRGEQLLLQIKQILDLTKADKVNLIGHSHGALTARYVAACYPELVASVTSVNGVNHGSEIADVMLKVLKNKLSSSIANKLISHFVNSVTLLSTKRHLPQDFIGALNCLSTEGVKHFNNQYPQGIPTTWGGEGLELENNNVYYYSWSGILNTIPITLSNKFSLLSLSSRYFVKELQQNDGLVGRFSSHLGKVIRSDYPMDHAAAVNQIRGKCNASIDPTALYIEHLQRLALKGL

SEQ ID NO: 15 - DNA, 867 bp, Pseudomonas sp.
  source 1..867: mol_type = genomic DNA; note = Pseudomonas sp. K2I15
atgagcaaagaagcgtcgactcaatatccaatggtgctcgttcacgggctcttcggatttgattccatcgccggctatccttattttttcaatattcagccggcacttgagagagccggtgcaaaggtatttacagtgaacattcccgcggtcaacggaaacgaagagcggggtgaaaagctgcttgaacaagtaaacttaatactgcagcaaacgggggcagccaaagtgaatctgatcggacattcacaaggacccctggcagctcgttatgtggctgcgattcatccggaaaaagttgccagtgtcacgtctgtttcctgcccgaatttcggcagtgagattgctgatcagcttcgcaaagcattaattcctggaacgcttccaaccgctgttgctgaagcaatcttaaacgctgtcggcatttttatttctttgatcagcggccatccaacaaatcctcaggatgcggcagcagcatttgaatcattaacaacagaaggccttgccgcttttaacctgaaatacccgcaaggcgttcctgctgtatggggcggagagggcaatgaagtggaaaacggtgtctactattacagctggtcagggatcgttcaggggtcgaagccgcagcttttagatttgagccatttgaactgtattgccctttccttattgttttataatgagaaaaatgcgaatgacggattggtaggccaaaacagctctcaccttggtaaagtcatcaaatcagattatccgatggatcattttgacgcagttaatcaacttgcaggtataactggctggaatgtcaatccggtgcagctgtacttagaccacgcagtgctgctaaagtctaaaggactc

SEQ ID NO: 16 - protein, 289 aa, Pseudomonas sp.
  source 1..289: note = Pseudomonas sp. K2I15
MSKEASTQYPMVLVHGLFGFDSIAGYPYFFNIQPALERAGAKVFTVNIPAVNGNEERGEKLLEQVNLILQQTGAAKVNLIGHSQGPLAARYVAAIHPEKVASVTSVSCPNFGSEIADQLRKALIPGTLPTAVAEAILNAVGIFISLISGHPTNPQDAAAAFESLTTEGLAAFNLKYPQGVPAVWGGEGNEVENGVYYYSWSGIVQGSKPQLLDLSHLNCIALSLLFYNEKNANDGLVGQNSSHLGKVIKSDYPMDHFDAVNQLAGITGWNVNPVQLYLDHAVLLKSKGL

SEQ ID NO: 17 - DNA, 864 bp, Arsenophonus nasoniae
  source 1..864: mol_type = genomic DNA
atgccgacaaaatacccaatcattttggtgcacggcctcttcggttttgataaaatcgccggatacccatgctttttcgccattgaaaaccgattaaagaaacaaggctataacgtattttcacccatattatccggtgtaaactcgaatgaagtgaacggcgagcagctttggctgtatatcgaggagttaaaacgcaatatcggctgtgaaaaagtgaatttaatagcccatagtcaaggagcgctgtttgctcgttatgtggcggcaaactattcagcatccattgcaagtgtaactagcatgaatggcgtaaatcacggttctgaaatcgctgatttggtcagaaaagtacttattcctgggaagctgacagaaacggttgtcgttacggctgctgaaatcttttttacatttatttctttaatttcatctggcacgctgaagcctcaggacggcgttgaagcattgaactcgctcaccactgaggttgttaacgaatttaataaaaaatatccgcaagggcttccgaaagaatggcggggagaaggagatgaagttgtgaacggagtgcattattacagcttcggcagctttatcaaaaagtccctgataaacagcggaatcaatgcgtttgacgtgtctcatacatcattactacagctgtcctctttcttcagtagggagaaggaaaatgacggacttgtcggccgctactcaatgagacttggaaaattgatttgcgatgattatgatatggatcatcttgatattgttaatcagattgccggggtcgtcagcaatcaatatgacattccgtcaatttatgtcaatcatgcgcaaatgctggcaaaaaaagggctc

SEQ ID NO: 18 - protein, 288 aa, Arsenophonus nasoniae
MPTKYPIILVHGLFGFDKIAGYPCFFAIENRLKKQGYNVFSPILSGVNSNEVNGEQLWLYIEELKRNIGCEKVNLIAHSQGALFARYVAANYSASIASVTSMNGVNHGSEIADLVRKVLIPGKLTETVVVTAAEIFFTFISLISSGTLKPQDGVEALNSLTTEVVNEFNKKYPQGLPKEWRGEGDEVVNGVHYYSFGSFIKKSLINSGINAFDVSHTSLLQLSSFFSREKENDGLVGRYSMRLGKLICDDYDMDHLDIVNQIAGVVSNQYDIPSIYVNHAQMLAKKGL

SEQ ID NO: 19 - DNA, 882 bp, Enterobacillus tribolii
  source 1..882: mol_type = genomic DNA
atgaaaaaagcaactacgcttaaatatccgattatcttggtgcacggactttttggttttgacaaaatcgctggcgtttatccttattttttcggtgtaaaagaagctcttgaaaaagcgggggcggaagtgtatgtcgcatcactgtcggcagtaaattcaaacgaagttcgcggtgagcagctcatggactttgtcaatgaggtgctggcaaataccggtgcaaagaaggtgaacttgatcggccactctcaaggcccgcttgcctgccgttacgtggctgcattacgccctgatattgttgcttctgtgacaagcgttcatggcgtcaacttcggcagcgagttagccgatgtggtccgtcaggccttgattccagggaggttgcctgaagcgatagctcatgcggtagtcacaacatttggagatttcttatcgctaatttcaggaaagccgatgcttgcgcaggatgcaaaagccgccttagacgcccttacctcagaaggaatcgcagaatttaatgcgaagtacccgcaagggctgccatctgaatggggaggagaaggcgatgaatatgtaaacggcgtatattattacagctggggcggagttttaaaatacaatatctttgatcagctgttgaacaatctggatcccacacatattgcgatgagtgctctttccattttctttaacaaagagcggggacaaaatgacggcgttgtcggtagatactctatgcatttaggaaaagttatacgatctgattattcaatggatcacctcgacgctgtaaatcaaacggcaggggttgtcacgactagtgtcaatccggtgaagctgtatgttgatcatttgtatcttctgagaagcaaaggcctc

SEQ ID NO: 20 - protein, 294 aa, Enterobacillus tribolii
MKKATTLKYPIILVHGLFGFDKIAGVYPYFFGVKEALEKAGAEVYVASLSAVNSNEVRGEQLMDFVNEVLANTGAKKVNLIGHSQGPLACRYVAALRPDIVASVTSVHGVNFGSELADVVRQALIPGRLPEAIAHAVVTTFGDFLSLISGKPMLAQDAKAALDALTSEGIAEFNAKYPQGLPSEWGGEGDEYVNGVYYYSWGGVLKYNIFDQLLNNLDPTHIAMSALSIFFNKERGQNDGVVGRYSMHLGKVIRSDYSMDHLDAVNQTAGVVTTSVNPVKLYVDHLYLLRSKGL

SEQ ID NO: 21 - DNA, 882 bp, Yersinia enterocolitica
  source 1..882: mol_type = genomic DNA
atgagcacgaacagcactttaaaatacccggttgtgttagttcacggcctgcttggttttgataagatcgccggtgtttatccatatttttacggcgttgaagaacctttgaaaaaagcgggcgcacaggtgtttgtcgcaaccatctccgctacaaactcaaatgaagtaagaggcgaacagcttttgaagtttgtgaaagaagtcatggcaaaaacaggagccaagaaagtgaacttgatcggccacagccaaggcccgctagcttgccgatatgtggcggcgactcatccggagcttattgcatctgtaacgtcagtaaacggggtcaatcacgggagtgagattgctgaccttgtcagatcggctttggtcccaggatcactccccgagcatattgtgaatacaattatgagtgctttcggagtattcgtttctcttttatccggaaaaccgttcctgcctcaggattttatggaaagcatcgacgcgctgaccacagaaaatgtcgcgaaatttaacacgaaatatccgcagggtcttcctgaaacgtgggggggcgaggggaaagaatttgacaatggcgtatattattacagctggggaggtgtccttggctataacccgctcattgaaggcttaaataatctggatccactccatcattctctcgtggccttatcgctgctgttcacaaaagaacgcaaccaaaatgacgggttagtcggtcggtactccatgcatttaggtaaagtcatacgttcagattatcaacttgatcatgttgatgccatcaatcaaacagcaggaatggtttcaaaggatatagatcctgttcaattatttgttaatcagattgaattgctgaagtctaaaggactg

SEQ ID NO: 22 - protein, 294 aa, Yersinia enterocolitica
MSTNSTLKYPVVLVHGLLGFDKIAGVYPYFYGVEEPLKKAGAQVFVATISATNSNEVRGEQLLKFVKEVMAKTGAKKVNLIGHSQGPLACRYVAATHPELIASVTSVNGVNHGSEIADLVRSALVPGSLPEHIVNTIMSAFGVFVSLLSGKPFLPQDFMESIDALTTENVAKFNTKYPQGLPETWGGEGKEFDNGVYYYSWGGVLGYNPLIEGLNNLDPLHHSLVALSLLFTKERNQNDGLVGRYSMHLGKVIRSDYQLDHVDAINQTAGMVSKDIDPVQLFVNQIELLKSKGL

SEQ ID NO: 23 - DNA, 882 bp, Escherichia sp.
  source 1..882: mol_type = genomic DNA; note = Escherichia sp. E1130
atgaagattcagacgcaattaaattaccctgtcgtgcttgtccacggcttgttcggttttgataaaattgcaggggtttatccgtatttttacggcatcaaagatgccttggaagaagctggggccaccgtgttcatcgcttctatttcagcagtaaatgacaatgagcttcggggagagcagctgcttgcatatatcaatgatgtgctgaaaaaaacaggaaaagagaaggttaacctcatcggccattcacaggggcctttggcttgccgctatgtggctgcaacacaccccacattagttgcctctgtcacttctgtaaacggtgtgaatttcggctcagagttcgcggacctcgttagatctgcgctcattccgggtgaaatccctgaagtcattgccaacagtatacttgacgtttttgcgaagctgctgacggccatctccggaaatccggattttccgcaggattcgatagctgcgctggatgcgctaacaacggaaggggtagcaaaatttaacgaaaaatatcctcaaggactcccgattgtacgcggcggtgaaggcaaagaatttgacaacggtgtatattattacagctggagcggcattatagacagcaatatcctgcatcaaggcatgaataactttgatccatctcatattgcgatgctcgcttgtagcatgctgtttgaaaatgaatatcatgaaaacgacggacttgtcggccgttatgcgtcccacttaggaaaggttatcagaagcgattattcgcttgatcatttggatgcaattaatcaaattgcaggagtgttgccacgatacagtgattcaatctccatttaccttgagcatttagagaggttaaaatcaaaaggatta

SEQ ID NO: 24 - protein, 294 aa, Escherichia sp.
  source 1..294: note = Escherichia sp. E1130
MKIQTQLNYPVVLVHGLFGFDKIAGVYPYFYGIKDALEEAGATVFIASISAVNDNELRGEQLLAYINDVLKKTGKEKVNLIGHSQGPLACRYVAATHPTLVASVTSVNGVNFGSEFADLVRSALIPGEIPEVIANSILDVFAKLLTAISGNPDFPQDSIAALDALTTEGVAKFNEKYPQGLPIVRGGEGKEFDNGVYYYSWSGIIDSNILHQGMNNFDPSHIAMLACSMLFENEYHENDGLVGRYASHLGKVIRSDYSLDHLDAINQIAGVLPRYSDSISIYLEHLERLKSKGL

SEQ ID NO: 25 - DNA, 879 bp, synthetic construct
  source 1..879: mol_type = other DNA
atgaatacagaagcgacaacaaaatacccaattgtgcttgttcatggtctattcggctttgataagatcgccggctacccttattttttcggtattaaggaggcacttgagaaggcgggagcaaaagtatttacgccttcaatatccgcagtcaactcaaatgaagtgaggggggagcagctgttagaacaggttcagcgaattctgaaaaaaacaggggctcaaaaagtgaatttaatcggtcacagccaagggccgctggcctgccgctatgtagctgcgatgcatccggaactggtcgcatctgtgacaagtgtctccggaccgaatcatgggagtgaaatcgcagatcagcttcggaaagcgctgaccccaggcgagttgcccgaggctgttgcatcaaccctgatgaacgcctttggaaactttatttctctcctttctggacaccctcagctcccgcaggatgctgtcgctgcattagatgccttgacgactgaaggcgttgctgaatttaacagaaaatatccacaaggccttcctgaaacatggggcggagaaggaaaagaaattgaaaacggagtatactattattcgtggagcggcattatcaaaggatcgattttggaccaaggattaaatacgcttgatccgcttcacttagcatgtcgcgcgctctcaaagctgttcactaaggaaaaaaatcaaaatgacggtctcgtaggaagatactccagccatttaggcaaagtcatccgttctgattatccgatggatcatttggatgccgtgaaccaaacggcgggtgtcgtttcaactaatgtagacccggtgaagctttatgttgaccatgcggctttattgaaaagcaaaggcttg

SEQ ID NO: 26 - protein, 293 aa, synthetic construct
MNTEATTKYPIVLVHGLFGFDKIAGYPYFFGIKEALEKAGAKVFTPSISAVNSNEVRGEQLLEQVQRILKKTGAQKVNLIGHSQGPLACRYVAAMHPELVASVTSVSGPNHGSEIADQLRKALTPGELPEAVASTLMNAFGNFISLLSGHPQLPQDAVAALDALTTEGVAEFNRKYPQGLPETWGGEGKEIENGVYYYSWSGIIKGSILDQGLNTLDPLHLACRALSKLFTKEKNQNDGLVGRYSSHLGKVIRSDYPMDHLDAVNQTAGVVSTNVDPVKLYVDHAALLKSKGL

SEQ ID NO: 27 - DNA, 870 bp, synthetic construct
  source 1..870: mol_type = other DNA
atgaatatggaagcgtcaacgcaatacccgatcgtgctggttcatgggttgttcggctttgataaaatcgccggctatccctattttttcggtataaaggaagcactggagagggcaggtgcaaaagtattcactgtaaacattcctgctgtcaacggcaacgaagaacgcggcgagaagttattagagcaagttaacagaattttacaaaaaacaggcgctgccaaggtgaacctgatcggccattctcaaggccctctcgcggcccgttacgtggctgcgcttcatccagagaaagttgcaagcgtcacaagcgtatcatgcccaaatcacggaagcgaaatagctgatcagctgcgaaaagcattaacgcctggcgagcttccggaggccgtggctctcgccctgcttaatgcggtcggtacttttatcagcctgatttctggacatccgcaaaacccgcaggatgcggcagctgcatttgaatctttaaccacagaagggcttgcggcctttaaccggaaatatcctcagggtgttcctgaaacatggggaggagaaggcaatgaaattgaaaatggcgtttattattactcctggtcaggaattgtgcagggatttcaatcactgcagccgcttgatccgtcgcacttgaactgtattgcccttagtaagctattttataaagaaaagaatgcaaatgacggtcttgtcggacagtattcgtcccacctcgggaaagtcatcagatctgattacccgatggatcattttgacgctgttaatcaaatggcggggattacgagctggaatgtaaatccagtaaaactctatttagaccatgcggcgttgttgaaaagtaaaggacta

SEQ ID NO: 28 - protein, 290 aa, synthetic construct
MNMEASTQYPIVLVHGLFGFDKIAGYPYFFGIKEALERAGAKVFTVNIPAVNGNEERGEKLLEQVNRILQKTGAAKVNLIGHSQGPLAARYVAALHPEKVASVTSVSCPNHGSEIADQLRKALTPGELPEAVALALLNAVGTFISLISGHPQNPQDAAAAFESLTTEGLAAFNRKYPQGVPETWGGEGNEIENGVYYYSWSGIVQGFQSLQPLDPSHLNCIALSKLFYKEKNANDGLVGQYSSHLGKVIRSDYPMDHFDAVNQMAGITSWNVNPVKLYLDHAALLKSKGL

SEQ ID NO: 29 - DNA, 879 bp, synthetic construct
  source 1..879: mol_type = other DNA
atgaaaacgacgactaccacaaaatacccgattgttctcgtacacggccttttcggctttgataaaatcgcaggctacccttatttttttaatattgatgaatcattaagaaaacaaggggcaacggtttttacaccggccatatcggcagcaaattccactgaaacacgcggagagcagcttttagcacaggtgaaaaagatcctgaagaagacgggcgcccaaaaggtcaatctgatcggccattctcagggtgcgctgacatgccgttatgtggctgcgcttcacccggagcttgtggcatccgtaacctcggtcaacggcgtgaatcatggaagcgaaatcgctgatttaatgctgaaagtgctgtccggtaagctgcccggtgctgttgcttcaaagattatgaacgcgtttatgaattttatttctctattgagcactaagccacagctcccgcaagactttgtctcagcgttaaacagcctgagcacagaaggggtcgctgaatttaacaaaaaatatcctcaggggcttccaaaaacatggggcggagaaggcaaagagcttgaaagcaacggagtttattactactcttggtcaggaatcattaaatcaaaaatattaaatgaaggattgaatacgttggacccatctcacgcgattcttgccgccttgtctaaattcttcaccaaagaaaaaaaccaaaatgacggcctcgtcggaaggttcagtagtcatttaggaaaagttatccggtccgattatccgatggatcatcttgatgcggtaaatcaaattgccggtgtatgttcaacaaatgttgaccctgtaaacctgtatattgagcatgcagctcgattaaaaagcaaagggctc

SEQ ID NO: 30 - protein, 293 aa, synthetic construct
MKTTTTTKYPIVLVHGLFGFDKIAGYPYFFNIDESLRKQGATVFTPAISAANSTETRGEQLLAQVKKILKKTGAQKVNLIGHSQGALTCRYVAALHPELVASVTSVNGVNHGSEIADLMLKVLSGKLPGAVASKIMNAFMNFISLLSTKPQLPQDFVSALNSLSTEGVAEFNKKYPQGLPKTWGGEGKELESNGVYYYSWSGIIKSKILNEGLNTLDPSHAILAALSKFFTKEKNQNDGLVGRFSSHLGKVIRSDYPMDHLDAVNQIAGVCSTNVDPVNLYIEHAARLKSKGL

SEQ ID NO: 31 - DNA, 864 bp, synthetic construct
  source 1..864: mol_type = other DNA
atgagcacgaaatatccgattgtgttagtacacggtttattcggttttgataaaatcgccggctatccttatttttttggaattaaagatgcactgaaaaaggcagggcataaagtatttacagcctccctctcggctgttaacagcaatgaagtgagaggcgagcagctgtgggaatttgtacaggaaatcctgaagaagacgggagctaaaaaagtgaacttgatcggtcacagtcaggggccccttgcatgccgctatgtcgcggccatgcatcctgaatcagtagcttctgttacttctgttaacggagtaaatcacggctcagaaattgcggacctcgtccggaaggtgctgacgccgggcagccttccggaagcagttgcgaacacagtcatgaatgccttcggcacgtttatttctctactatccggacatccgcaaaaacctcaggatgccgtcgctgcgcttgaggcgttaaccacagaaggcgtaaccgagtttaataaaaaatacccacaagggcttccaaaaacatggggaggagaaggaaaagagatcgtgaacggcgttcattattactcttttgggtcgttcattaaaggaagcatattagatcaaggcctgaatatgttggacccgactcatttggcaatgagagctttgagtaaatttttcacaaaagaaaaacaaaatgacggattagtcggccgttattcaatgaggctgggtaagctgatacgagatgattacagcatggatcatcttgatatggtgaatcaagtggcgggtgttgtttcaacaaacgttgacatcgtcaagatttatgtgaatcatgcaaagcttttagcatcaaaaggcctc

SEQ ID NO: 32 - protein, 288 aa, synthetic construct
MSTKYPIVLVHGLFGFDKIAGYPYFFGIKDALKKAGHKVFTASLSAVNSNEVRGEQLWEFVQEILKKTGAKKVNLIGHSQGPLACRYVAAMHPESVASVTSVNGVNHGSEIADLVRKVLTPGSLPEAVANTVMNAFGTFISLLSGHPQKPQDAVAALEALTTEGVTEFNKKYPQGLPKTWGGEGKEIVNGVHYYSFGSFIKGSILDQGLNMLDPTHLAMRALSKFFTKEKQNDGLVGRYSMRLGKLIRDDYSMDHLDMVNQVAGVVSTNVDIVKIYVNHAKLLASKGL

SEQ ID NO: 33 - DNA, 882 bp, synthetic construct
  source 1..882: mol_type = other DNA
atgaaaacgtccacgacgctgaagtatccgattgttctcgttcatggtctctttggctttgataaaatagctgggatttatccttatttcttcgggattaaagaggcgctggagaaggcaggtgcaaaagtgtttaccgcatccatttcggctgtaaacagcaatgaagtccgaggagaacagcttcttgagtttgtcaaagaggtacttgctaaaacaggagcaaaaaaggtgaatctgatcggtcacagtcaaggcccactggcctgccgctatgtcgcggccatgcatcctgagttggttgcctcagttacctctgttaacggtgtcaatcatggcagtgaaatcgcagatcttgtcagaaaagctttaacaccaggctctcttccggaagcgatcgctaatacagtcatgaatgcgttcggaaattttctttcactgatttcggggcatccgcagctgccgcaagatgctgttgcggccttagatgcactaacaactgaaggtgtagcagaattcaacgctaagtaccctcagggccttcctgaaacatggggaggcgaaggaaaagaatttgaaaacggcgtttactattatagctggggcggaatcatcaaatacaacattttagaccaaggattgaacaaccttgatccgcttcacattgcaatgagagcgttatctttgttttttacaaaagaacggaatcaaaatgatgggctcgtgggcaggtacagcatgcacttgggtaaggtcatacgttctgattattcaatggatcatctggacgcggtgaatcagactgccggagtggtcagcacgaatgtggaccccgtaaagctgtatgtagaccatgtggccctcttgaaatcaaaaggatta

SEQ ID NO: 34 - protein, 294 aa, synthetic construct
MKTSTTLKYPIVLVHGLFGFDKIAGIYPYFFGIKEALEKAGAKVFTASISAVNSNEVRGEQLLEFVKEVLAKTGAKKVNLIGHSQGPLACRYVAAMHPELVASVTSVNGVNHGSEIADLVRKALTPGSLPEAIANTVMNAFGNFLSLISGHPQLPQDAVAALDALTTEGVAEFNAKYPQGLPETWGGEGKEFENGVYYYSWGGIIKYNILDQGLNNLDPLHIAMRALSLFFTKERNQNDGLVGRYSMHLGKVIRSDYSMDHLDAVNQTAGVVSTNVDPVKLYVDHVALLKSKGL

SEQ ID NO: 35 - DNA, 882 bp, synthetic construct
  source 1..882: mol_type = other DNA
atgagtacaagcacgacgctgaagtatccgattattttagttcatggattttccggctttgataaaatcgcaggcatttatccttatttttatggtattcagcaggcgctcgagaaagcaggtgcaacagtattcaccgcatctatttctgcggaaaattcaaatgaagtgcgaggtgaacagcttcttgaatttgtcaaacaagtgatcgccttgaccggcgctgaaaaagttaatctgatcggacattcacaagggccgctggcttgccgctatgtagctgctatgcatccggagctggttgcctcggtaacgtctgtgaacggcgtcaacttcggttctgaaatcgctgacttagtacggctcgcagtgaagcccggaagcctgccagaagcgattgcatccacggtcatgaatgccttcggcagctttttatccctcattacagggcatccttcgctgcctcaggacagtgtggcggccttagatgctctcacttcagaaggagtcgcaaaatttaatgcgaaatacccgcaagggcttccgtcaacatggggcggagaaggcaaggagtttgaaaacggggtttattattacagctggggaggaatcataaactacaaccctcttgatcaaggcttaaataacttagacccacttcacactgcgatggttgcgctttctctgttgttcacaaaagagagatttcaaaatgatggacttgtcgggcgttacagcatgcacttgggaaaagtgataaggagcgattattcaatggatcatttggacgccattaatcaaacagctggtgttgtcacttctgatgccgatccggttcagctgtttgttgaccacgtggcgagattgaagtcaaaaggcctt

SEQ ID NO: 36 - protein, 294 aa, synthetic construct
MSTSTTLKYPIILVHGFSGFDKIAGIYPYFYGIQQALEKAGATVFTASISAENSNEVRGEQLLEFVKQVIALTGAEKVNLIGHSQGPLACRYVAAMHPELVASVTSVNGVNFGSEIADLVRLAVKPGSLPEAIASTVMNAFGSFLSLITGHPSLPQDSVAALDALTSEGVAKFNAKYPQGLPSTWGGEGKEFENGVYYYSWGGIINYNPLDQGLNNLDPLHTAMVALSLLFTKERFQNDGLVGRYSMHLGKVIRSDYSMDHLDAINQTAGVVTSDADPVQLFVDHVARLKSKGL

SEQ ID NO: 37 - DNA, 882 bp, synthetic construct
  source 1..882: mol_type = other DNA
atgtcaacatctaccactttaaaatatccgattgttctagtccatggattattcggatttgataaaattgccgggatctatccatatttttacggaataaaggaagcacttgaaaaagctggagccacagtatttaccgcatcaataagtgctgttaacagcaatgaagtgagaggtgaacagcttttggagtttgtaaaagaggtgctggccaaaacaggcgcggaaaaggtaaacctcatcggccattcacaaggacctctggcttgccgctatgtagcggcaacgcacccagagctggtggctagcgtcacgtcagtcaatggcgtgaatcacggcagtgaaattgctgatcttgttcgttccgcattgaaaccgggttcgctccctgaagcaattgccaacacggtgatgaatgctttcggacaatttttatctgcgatttcagggcatccgcagctgccccaagactcggttgcggcccttgatgcgctgacgactgaaggagttgccaaatttaacgcgaagtaccctcagggcctgccggccacatggggcggagagggcaaggaatttgacaacggcgtgtattactatagctggtccggaatcatcaactacaatccgctcaatcaagggttaaataatctggaccctttgcatattgcaatggttgcccttagcctattgtttacaaaagaacggttccaaaacgacggtttagtaggtagatactccagccatctggggaaagtcattaggtcagattattctatggatcaccttgatgctatcaatcagacagcgggtgtcgtgtcctctgacgctgatccggttaagttgtatgtcgatcatgtcgcacgattgaaatctaaaggcctt

SEQ ID NO: 38 - protein, 294 aa, synthetic construct
MSTSTTLKYPIVLVHGLFGFDKIAGIYPYFYGIKEALEKAGATVFTASISAVNSNEVRGEQLLEFVKEVLAKTGAEKVNLIGHSQGPLACRYVAATHPELVASVTSVNGVNHGSEIADLVRSALKPGSLPEAIANTVMNAFGQFLSAISGHPQLPQDSVAALDALTTEGVAKFNAKYPQGLPATWGGEGKEFDNGVYYYSWSGIINYNPLNQGLNNLDPLHIAMVALSLLFTKERFQNDGLVGRYSSHLGKVIRSDYSMDHLDAINQTAGVVSSDADPVKLYVDHVARLKSKGL

SEQ ID NO: 39 - DNA, 882 bp, synthetic construct
  source 1..882: mol_type = other DNA
atgagcacttcaactacgctgaagtacccgattgttcttgtccacggtttgttcggatttgataaaatcgcgggtatttatccttatttttacggcatcaaggaggcgttagaaaaagccggcgcaaccgtgttcacggcatcaatcagcgctgtaaattctaatgaggtacgcggagaacagttgcttgaatttgtgaaagaagtgcttgcaaaaacaggcgccaaaaaagtgaacctcattggacattctcaaggcccgcttgcctgccgttatgtggccgcgatgcatccagagctcgtggcttctgttacatccgtcaacggtgtcaatcatgggtccgaaatcgctgatctcgtaagatcggcgctgacaccgggatcgctgcctgaagcaattgcgaacaccgtcatgaatgcgttcggtaactttttgagcctaataagtgggcatccacagctgcctcaggactcagtagcagcacttgacgctttaacaactgaaggagttgctaaatttaatgccaaatatccccaggggctgccagaaacatggggcggcgaaggcaaggagtttgaaaatggggtttattattacagctgggggggcataattaactataatccgctggatcaaggattaaacaatttagaccctcttcatattgcaatggttgcgttgtctctgttatttacaaaagagagaaaccaaaatgatggactagtcggcaggtattcaatgcacttgggaaaagtcattcggagtgactacagcatggatcaccttgatgccatcaatcaaacggcaggtgttgtatcctctgatgtggatccggttaagctgtatgtcgaccatgttgctttactaaagtcaaaaggattg

SEQ ID NO: 40 - protein, 294 aa, synthetic construct
MSTSTTLKYPIVLVHGLFGFDKIAGIYPYFYGIKEALEKAGATVFTASISAVNSNEVRGEQLLEFVKEVLAKTGAKKVNLIGHSQGPLACRYVAAMHPELVASVTSVNGVNHGSEIADLVRSALTPGSLPEAIANTVMNAFGNFLSLISGHPQLPQDSVAALDALTTEGVAKFNAKYPQGLPETWGGEGKEFENGVYYYSWGGIINYNPLDQGLNNLDPLHIAMVALSLLFTKERNQNDGLVGRYSMHLGKVIRSDYSMDHLDAINQTAGVVSSDVDPVKLYVDHVALLKSKGL

SEQ ID NO: 41 - DNA, 882 bp, synthetic construct
  source 1..882: mol_type = other DNA
atgaaaagtaatacacagacgaagtatccgatcgttctcgtgcacgggctttttgggtttgataaaatcgcgggctacccttattttttcggcattgcagaagctttaagaaagcaaggagcacaggtattcacagcttccgtcagtgccgtgaacagcacagaagttcggggagagcagttattggctcaagtaaaggaaattttaaaaaaaactggtgccgaaaaagtgaacctgatcgggcattctcagggtgcgccgacttgcaggtacgttgcggctgttcatccggagctggtggcatcagttacgtccgtaaacggtgtaaatcatggctcggagattgctgatttgcttcgaaaggtgctttctccaggttcattagccgaagcagttgccgctgcgattgtcaatgcatttggaaattttatttccttactaagtggcaacccgcagctgcctcaggacgcaatcggcgcattggattcgttgacgaccgaaggtgtagctgaatttaatcaaaaatatccccaaggtctcccaaaaacgtggggaggcgagggagctgagtttgaagtgaacggtgtctattattacagctggagcgggataataaaaaacggcctattaaatgaaggcctgaataccctggatccgtctcacgccctccttgcagtgcttagcaaattctttacaaaagaagcggaacaaaatgacggacttgtcggacgttactcatctcatctcggaaaagtcattcgcagcgattatcaaatggaccaccttgatgccatcaatcaaatggcgggaattcattcaacaaatgttgaccctgtcaacctttatgttgagcatgcagcgagactgaagtcaaaaggcctg

SEQ ID NO: 42 - protein, 294 aa, synthetic construct
MKSNTQTKYPIVLVHGLFGFDKIAGYPYFFGIAEALRKQGAQVFTASVSAVNSTEVRGEQLLAQVKEILKKTGAEKVNLIGHSQGAPTCRYVAAVHPELVASVTSVNGVNHGSEIADLLRKVLSPGSLAEAVAAAIVNAFGNFISLLSGNPQLPQDAIGALDSLTTEGVAEFNQKYPQGLPKTWGGEGAEFEVNGVYYYSWSGIIKNGLLNEGLNTLDPSHALLAVLSKFFTKEAEQNDGLVGRYSSHLGKVIRSDYQMDHLDAINQMAGIHSTNVDPVNLYVEHAARLKSKGL

SEQ ID NO: 43 - DNA, 879 bp, synthetic construct
  source 1..879: mol_type = other DNA
atgaaaacgaatacgactaccaaatacccgattgttctagttcacggcttgttcggctttgataaaatcgcaggctatccttatttctttggaattaaggaagcattagaaaaagcaggtgcacaggtttttacggctagtgtttctgctgttaacagcaatgaagtgcggggagaacaactgctcgaacaggtgaaggagattctgaaaaaaaccggggctgagaaggtgaaccttataggccattcgcaaggcgccttaacctgcaggtatgtcgcagccattcatccggaacttgtagcctctgtcacgtccgtaaacggagtgaatcatggttcagaaatcgctgatttgttgagaaaagcgcttacaccaggtagtttaccagaagccgtggcggcggctgtcgtatccgcctttggcaattttatttcacttttatctggaaaccctcagctgcctcaagatgcgattgccgcgttagacgcgctgactacagaaggcgttgctgaatttaaccaaaaatatccgcaggggctgccgaaaacatggggcggcgaaggagcagaggttgtcaatggtgtatattattacagctggtcaggcattatcaaaaacgggcttttgaatcagggactcaatacacttgaccccacacatgcggcaatgagagtgctgagcaaatttttcacaaaagaagcggagcaaaatgacggtcttgtcgggcgttactcaagccacctcggaaaggtaatacgatctgattattccatggaccacttagatgcaatcaatcaaatggctggaatcgtcagcacaaacgttgatccggtaaagctctacgtggagcatgcagcgcgccttaagtcgaaaggactg

SEQ ID NO: 44 - protein, 293 aa, synthetic construct
MKTNTTTKYPIVLVHGLFGFDKIAGYPYFFGIKEALEKAGAQVFTASVSAVNSNEVRGEQLLEQVKEILKKTGAEKVNLIGHSQGALTCRYVAAIHPELVASVTSVNGVNHGSEIADLLRKALTPGSLPEAVAAAVVSAFGNFISLLSGNPQLPQDAIAALDALTTEGVAEFNQKYPQGLPKTWGGEGAEVVNGVYYYSWSGIIKNGLLNQGLNTLDPTHAAMRVLSKFFTKEAEQNDGLVGRYSSHLGKVIRSDYSMDHLDAINQMAGIVSTNVDPVKLYVEHAARLKSKGL

SEQ ID NO: 45 - DNA, 879 bp, synthetic construct
  source 1..879: mol_type = other DNA
atgaaaacaaacacaacgacaaagtacccgattgttctcgttcatggattattcggttttgataaaatagccggctatccttattttttcggaatcaaagaagcgcttgaaaaagcaggggcacaagtgtttacggcttctgtttctgcggtaaactcgaatgaagtaagaggagagcagttgcttgagtttgtcaaagagattttgaaaaaaacgggtgccaaaaaggtgaacctgatcggccacagccaaggcccgctggcatgccgttacgtggctgcgatgcaccccgagcttgtcgcttccgtcacaagcgtgaatggcgtaaatcatggcagtgaaatcgcagatttggtccgaaaagcgctcaccccaggaagccttcctgaagccgttgcgaacgctgttgtaagtgctttcggcaattttatttcgcttctgtccggaaatccgcagctgcctcaggatgcgattgcggctttagacgcattaaccactgaaggcgtggccgaatttaatgcaaaatatccgcaagggttgccaaagacatggggaggagagggtaaggaagtggtcaacggtgtgtattattactcatggggcggcatcattaaaaacgggattttaaatcaagggctgaacacgcttgatccgactcatattgcaatgagagtgctgtctaaattttttacaaaagaagcagaacaaaatgacggactcgtcggccgctacagcatgcatttaggaaaagtaataaggtctgattattcaatggatcatttagacgccatcaatcagactgcaggtgttgtctcaacaaatgttgaccctgttaagctgtatgttgatcacgctgcccggctaaaatcaaagggactc

SEQ ID NO: 46 - protein, 293 aa, synthetic construct
MKTNTTTKYPIVLVHGLFGFDKIAGYPYFFGIKEALEKAGAQVFTASVSAVNSNEVRGEQLLEFVKEILKKTGAKKVNLIGHSQGPLACRYVAAMHPELVASVTSVNGVNHGSEIADLVRKALTPGSLPEAVANAVVSAFGNFISLLSGNPQLPQDAIAALDALTTEGVAEFNAKYPQGLPKTWGGEGKEVVNGVYYYSWGGIIKNGILNQGLNTLDPTHIAMRVLSKFFTKEAEQNDGLVGRYSMHLGKVIRSDYSMDHLDAINQTAGVVSTNVDPVKLYVDHAARLKSKGL

SEQ ID NO: 47 - DNA, 882 bp, synthetic construct
  source 1..882: mol_type = other DNA
atgagtacaaacacgacgctgaaatatccgattgtgcttgttcacggtctgttcggttttgataaaatcgctggaatttatccttatttttatggcattaaagaagcccttgaaaaagcgggcgcaactgtttttgtcgcgacgatttctgctgtaaacagcaatgaagtgagaggagaacaattattagaattcgtgaaagaggtacttgctaaaacaggcgccaaaaaagtaaatttgatcggacactcccagggcccacttgcgtgccgctatgtcgctgcaactcacccggagctcatagcctctgtcacctcagtgaacggcgtcaatcatggttcagaaatcgcagacctggtaaggtcggcgctgacacctggttccctgccggaagccatagcgaatacagtcatgtcagcattcggacaatttttatcactgctcagtggaaatccgcagcttcctcaggattccattgaagctttggacgcattgacgacagagggggtggcaaagtttaatgcgaagtacccgcaaggactcccaagcacatggggaggcgaaggcaaggaatttgacaacggagtatattattacagctggggcgggatcatcaattacaaccccctgaatcaggggttaaacaaccttgatccgctgcatattgcaatggttgccttgagtctattgtttacaaaggagcgttttcaaaatgatgggcttgtcggcagatactcaatgcatttaggaaaagtcattcgctctgactatagcatggatcatgttgatgcgattaatcaaaccgcaggtgttgtttcttcggatgctgatcctgttaagctttatgtggaccatatcgcccggttaaaaagcaaagggttg

SEQ ID NO: 48 - protein, 294 aa, synthetic construct
MSTNTTLKYPIVLVHGLFGFDKIAGIYPYFYGIKEALEKAGATVFVATISAVNSNEVRGEQLLEFVKEVLAKTGAKKVNLIGHSQGPLACRYVAATHPELIASVTSVNGVNHGSEIADLVRSALTPGSLPEAIANTVMSAFGQFLSLLSGNPQLPQDSIEALDALTTEGVAKFNAKYPQGLPSTWGGEGKEFDNGVYYYSWGGIINYNPLNQGLNNLDPLHIAMVALSLLFTKERFQNDGLVGRYSMHLGKVIRSDYSMDHVDAINQTAGVVSSDADPVKLYVDHIARLKSKGL

SEQ ID NO: 49 - DNA, 879 bp, synthetic construct
  source 1..879: mol_type = other DNA
atgaatacaaatgcgacgacgcagtacccgattgtgctcgtccacggattgttcggctttgaccgcattgccggttatccttatttttacggcattaaacaggctcttgaaaaagcaggtgcgcaagtgttcaccgcaagcgtttctgctgtgcacagcaatgaggtgaggggagagcagctgctggaacaaattgaacgaatcttgcggcagacaggtgcagaaaaggtcaatctaatcggacattcacaaggagcgctgactgcaagatacgcagccgctatacgccccgaacgggtggcttctgtcacctctgtatccggtccgaatcatggcagtgagctggctgatttattaagaaaagcactgacccctggctccttgccagaggcagttgcagctgcgcttgtcactgcgtttgcaaactttatgagtcttctcagcggaaacccgcagctccctcaggatgcgatcgccgcattagatgctttaacaacagaaggagttgccgcctttaatcaaaaatacccgcaagggctgccaaaaacatggggaggggaaggcgctgaacaggtgaacggcgttcattattattcgtggtccggcattattcaagggggtctgttaaatcagggattgaaccttctggacccgacgcatgcggcctgccgcgttctaagccgtttttttacaagagaagcggagcaaaacgacggcatggtcggaagattctcttcacaccttggaaaagtcatccgttcagattatccgatggatcatctcgacacgataaaccaaatggcggggcttgtatcaaaaaatgttgatcctgtaaagctttatgtagaacatgctgcccgtttaaaatcaaagggtctc

SEQ ID NO: 50 - protein, 293 aa, synthetic construct
MNTNATTQYPIVLVHGLFGFDRIAGYPYFYGIKQALEKAGAQVFTASVSAVHSNEVRGEQLLEQIERILRQTGAEKVNLIGHSQGALTARYAAAIRPERVASVTSVSGPNHGSELADLLRKALTPGSLPEAVAAALVTAFANFMSLLSGNPQLPQDAIAALDALTTEGVAAFNQKYPQGLPKTWGGEGAEQVNGVHYYSWSGIIQGGLLNQGLNLLDPTHAACRVLSRFFTREAEQNDGMVGRFSSHLGKVIRSDYPMDHLDTINQMAGLVSKNVDPVKLYVEHAARLKSKGL

SEQ ID NO: 51 - DNA, 879 bp, synthetic construct
  source 1..879: mol_type = other DNA
atgcagagaaatgcaactactcaatatccgatacttctcgttcacggccttttcggctttgatcggatcgggaaatttgaactctttcatggaatcaaacaggcgcttcgcaatgccggtgcaagggtatttgtcccttatctctctgctgttcactccaatgaagtgcgaggagaacagctccttgcccaaattgaccgtgtgctggcggaaacaggagcttcaaaagtgaatctgatcgggcattctcaaggcgctttagctgccagatacgctgcagccattcagcctgagcgggttgcaagtgtgacaagcgttagtgggccaaatcatggttcggagttggctgattatcttaggaaagcgctaacacctggacaattgcccgagcatgtagcggctgccgtcacaacgctgtttgctgaatttttatcattgctaagcggcaatccgcagcttccgcaaaacgcgattgcagcgctgaacgccttgacgacggaaggcgtagccgcatttaaccaaaaatatcctcagggtctgccgaaaacatggggaggaaatggaaaggaacaagtgaacggcgtccgctattacagctggtcaggcattttgcagggaaaccttctggatgaaggattaaacttacttgatccactgcatgcggcatgccgcgctttctcccggttcttcacaaccgaggcggagcaaaatgacggcatggtcgggcgtttttcaagccacttagggaaggtcattcgttctgattacccgatggaccatatggatacgatcaatcaaaccgcaggtttagtcagaaaaggcgttgacccggtagaactttatgttcagcatgcagaaagactgaagtctgttggtttg

SEQ ID NO: 52 - protein, 293 aa, synthetic construct
MQRNATTQYPILLVHGLFGFDRIGKFELFHGIKQALRNAGARVFVPYLSAVHSNEVRGEQLLAQIDRVLAETGASKVNLIGHSQGALAARYAAAIQPERVASVTSVSGPNHGSELADYLRKALTPGQLPEHVAAAVTTLFAEFLSLLSGNPQLPQNAIAALNALTTEGVAAFNQKYPQGLPKTWGGNGKEQVNGVRYYSWSGILQGNLLDEGLNLLDPLHAACRAFSRFFTTEAEQNDGMVGRFSSHLGKVIRSDYPMDHMDTINQTAGLVRKGVDPVELYVQHAERLKSVGL

SEQ ID NO: 53 - DNA, 888 bp, synthetic construct
  source 1..888: mol_type = other DNA
atgagcacaaacgccagaacccgctacccgttagtgcttgttcacgggttgctgggctttgtcaggattgccggctacccatattggtatggaatcacatcggcgctggaaagggcgggcgcgcaggtatacccagtgcgggtgtcagctgtccacagtaatgaagtcagaggggagcagcttttagagcaaattgaacgaatattacgccaaaccggtgctgagcgtgtaaaccttatcggccattcacaaggagcactcacggcacgctatgctgccgcgattcgaccagaaagagtcgcgtcagtaacttcagttgcggggcccaatcatggaagtgagctggctgatatgctgcaaagaagcctccccccgggttctcttcgggaacagctcgctgcgtctctagttcaggcccttgcgaagtttatggctttcttagaccgtgcagaccggtcaccgcgtctgcctcaggatgcattggcttctcatgaagccttaacgactgaaggggtagcagcatttaatgcaaaatatccgcaaggccttcctgaaacatggggaggagagggcgcagctgaagtgaacggcgttcattattacagctggtccggcattctgcagccgggattgacggacagaggtgccaaccggcttgatccgacacatgccatgtgcagaaggctgtcgcgctgttttacaagagaagcggaacaaaatgacggtatggtgggccgtttcagctcccacctcggaaaagtgattcgttctgattatcctttagatcatttggatatcatcaatcaaatggcgggtgcagtcgggcagggagttgatcctgtcgcattgtatgttgagcatgcagcccgcctgaaagaagcaggactc

SEQ ID NO: 54 - protein, 296 aa, synthetic construct
MSTNARTRYPLVLVHGLLGFVRIAGYPYWYGITSALERAGAQVYPVRVSAVHSNEVRGEQLLEQIERILRQTGAERVNLIGHSQGALTARYAAAIRPERVASVTSVAGPNHGSELADMLQRSLPPGSLREQLAASLVQALAKFMAFLDRADRSPRLPQDALASHEALTTEGVAAFNAKYPQGLPETWGGEGAAEVNGVHYYSWSGILQPGLTDRGANRLDPTHAMCRRLSRCFTREAEQNDGMVGRFSSHLGKVIRSDYPLDHLDIINQMAGAVGQGVDPVALYVEHAARLKEAGL

SEQ ID NO: 55 - DNA, 99 bp, Bacillus subtilis
  source 1..99: mol_type = genomic DNA
atgtttgcaaaacgattcaaaacctctttactgccgttattcgctggatttttattgctgtttcatttggttctggcaggaccggcggctgcgagtgct

SEQ ID NO: 56 - protein, 33 aa, Bacillus subtilis
MFAKRFKTSLLPLFAGFLLLFHLVLAGPAAASA

SEQ ID NO: 57 - protein, 11 aa, synthetic construct
  VARIANT 1: note = H
  VARIANT 2: note = A
  VARIANT 3: note = V, M, or I
  VARIANT 4: note = S, A, or Q
  VARIANT 5: note = X can be any amino acid
  VARIANT 6: note = X can be any amino acid
  VARIANT 7: note = R, P, or C
  VARIANT 8: note = C, D, or R
  VARIANT 9: note = E, S, A, or D
  VARIANT 10: note = X can be any amino acid
QGLPXXWGGXG